European Patent Application EP 4 656 655 A1, published December 3, 2025. Title: TCR MOLECULES TARGETING KRAS MUTATION, CELLS AND USE OF TCR MOLECULES AND CELLS. Applicant: BEIJING DCTY BIOTECH CO., LTD. The sequence listing filed with the application follows.

SEQUENCE LISTING (162 sequences)

SEQ ID NO: 1 - protein, 10 aa, synthetic construct
VVVGADGVGK

SEQ ID NO: 2 - protein, 10 aa, synthetic construct
KLVVVGAVGV

SEQ ID NO: 3 - protein, 278 aa, synthetic construct
MLTASLLRAVIASICVVSSMAQKVTQAQTEISVVEKEDVTLDCVYETRDTTYYLFWYKQPPSGELVFLIRRNSFDEQNEISGRYSWNFQKSTSSFNFTITASQVVDSAVYFCALSEVTGAGSYQLTFGKGTKLSVIPNIQNPDPAVYQLRDSKSSDKSVCLFTDFDSQTNVSQSKDSDVYITDKTVLDMRSMDFKSNSAVAWSNKSDFACANAFNNSIIPEDTFFPSPESSCDVKLVEKSFETDTNLNFQNLSVIGFRILLLKVAGFNLLMTLRLWSS

SEQ ID NO: 4 - protein, 117 aa, synthetic construct
AQKVTQAQTEISVVEKEDVTLDCVYETRDTTYYLFWYKQPPSGELVFLIRRNSFDEQNEISGRYSWNFQKSTSSFNFTITASQVVDSAVYFCALSEVTGAGSYQLTFGKGTKLSVIP

SEQ ID NO: 5 - protein, 7 aa, synthetic construct
TRDTTYY

SEQ ID NO: 6 - protein, 8 aa, synthetic construct
RNSFDEQN

SEQ ID NO: 7 - protein, 14 aa, synthetic construct
ALSEVTGAGSYQLT

SEQ ID NO: 8 - protein, 311 aa, synthetic construct
MSNQVLCCVVLCFLGANTVDGGITQSPKYLFRKEGQNVTLSCEQNLNHDAMYWYRQDPGQGLRLIYYSQIVNDFQKGDIAEGYSVSREKKESFPLTVTSAQKNPTAFYLCASSIGAGQHNSPLHFGNGTRLTVTEDLNKVFPPEVAVFEPSEAEISHTQKATLVCLATGFFPDHVELSWWVNGKEVHSGVSTDPQPLKEQPALNDSRYCLSSRLRVSATFWQNPRNHFRCQVQFYGLSENDEWTQDRAKPVTQIVSAEAWGRADCGFTSVSYQQGVLSATILYEILLGKATLYAVLVSALVLMAMVKRKDF

SEQ ID NO: 9 - protein, 115 aa, synthetic construct
DGGITQSPKYLFRKEGQNVTLSCEQNLNHDAMYWYRQDPGQGLRLIYYSQIVNDFQKGDIAEGYSVSREKKESFPLTVTSAQKNPTAFYLCASSIGAGQHNSPLHFGNGTRLTVT

SEQ ID NO: 10 - protein, 5 aa, synthetic construct
LNHDA

SEQ ID NO: 11 - protein, 6 aa, synthetic construct
SQIVND

SEQ ID NO: 12 - protein, 14 aa, synthetic construct
ASSIGAGQHNSPLH

SEQ ID NO: 13 - protein, 275 aa, synthetic construct
MLTASLLRAVIASICVVSSMAQKVTQAQTEISVVEKEDVTLDCVYETRDTTYYLFWYKQPPSGELVFLIRRNSFDEQNEISGRYSWNFQKSTSSFNFTITASQVVDSAVYFCALSEGSNYKLTFGKGTLLTVNPNIQNPDPAVYQLRDSKSSDKSVCLFTDFDSQTNVSQSKDSDVYITDKTVLDMRSMDFKSNSAVAWSNKSDFACANAFNNSIIPEDTFFPSPESSCDVKLVEKSFETDTNLNFQNLSVIGFRILLLKVAGFNLLMTLRLWSS

SEQ ID NO: 14 - protein, 114 aa, synthetic construct
AQKVTQAQTEISVVEKEDVTLDCVYETRDTTYYLFWYKQPPSGELVFLIRRNSFDEQNEISGRYSWNFQKSTSSFNFTITASQVVDSAVYFCALSEGSNYKLTFGKGTLLTVNP

SEQ ID NO: 15 - protein, 7 aa, synthetic construct
TRDTTYY

SEQ ID NO: 16 - protein, 8 aa, synthetic construct
RNSFDEQN

SEQ ID NO: 17 - protein, 11 aa, synthetic construct
ALSEGSNYKLT

SEQ ID NO: 18 - protein, 313 aa, synthetic construct
MGTRLLCWAALCLLGAELTEAGVAQSPRYKIIEKRQSVAFWCNPISGHATLYWYQQILGQGPKLLIQFQNNGVVDDSQLPKDRFSAERLKGVDSTLKIQPAKLEDSAVYLCASSSTGGTGETQYFGPGTRLLVLEDLKNVFPPEVAVFEPSEAEISHTQKATLVCLATGFYPDHVELSWWVNGKEVHSGVSTDPQPLKEQPALNDSRYCLSSRLRVSATFWQNPRNHFRCQVQFYGLSENDEWTQDRAKPVTQIVSAEAWGRADCGFTSESYQQGVLSATILYEILLGKATLYAVLVSALVLMAMVKRKDSRG

SEQ ID NO: 19 - protein, 115 aa, synthetic construct
EAGVAQSPRYKIIEKRQSVAFWCNPISGHATLYWYQQILGQGPKLLIQFQNNGVVDDSQLPKDRFSAERLKGVDSTLKIQPAKLEDSAVYLCASSSTGGTGETQYFGPGTRLLVL

SEQ ID NO: 20 - protein, 5 aa, synthetic construct
SGHAT

SEQ ID NO: 21 - protein, 6 aa, synthetic construct
FQNNGV

SEQ ID NO: 22 - protein, 13 aa, synthetic construct
ASSSTGGTGETQY

SEQ ID NO: 23 - protein, 271 aa, synthetic construct
MSLSSLLKVVTASLWLGPGIAQKITQTQPGMFVQEKEAVTLDCTYDTSDPSYGLFWYKQPSSGEMIFLIYQGSYDQQNATEGRYSLNFQKARKSANLVISASQLGDSAMYFCVGNEKLTFGTGTRLTIIPNIQNPDPAVYQLRDSKSSDKSVCLFTDFDSQTNVSQSKDSDVYITDKTVLDMRSMDFKSNSAVAWSNKSDFACANAFNNSIIPEDTFFPSPESSCDVKLVEKSFETDTNLNFQNLSVIGFRILLLKVAGFNLLMTLRLWSS

SEQ ID NO: 24 - protein, 110 aa, synthetic construct
AQKITQTQPGMFVQEKEAVTLDCTYDTSDPSYGLFWYKQPSSGEMIFLIYQGSYDQQNATEGRYSLNFQKARKSANLVISASQLGDSAMYFCVGNEKLTFGTGTRLTIIP

SEQ ID NO: 25 - protein, 7 aa, synthetic construct
TSDPSYG

SEQ ID NO: 26 - protein, 8 aa, synthetic construct
QGSYDQQN

SEQ ID NO: 27 - protein, 7 aa, synthetic construct
VGNEKLT

SEQ ID NO: 28 - protein, 311 aa, synthetic construct
MGSRLLCWVLLCLLGAGPVKAGVTQTPRYLIKTRGQQVTLSCSPISGHRSVSWYQQTPGQGLQFLFEYFSETQRNKGNFPGRFSGRQFSNSRSEMNVSTLELGDSALYLCASSLATGGYNSPLHFGNGTRLTVTEDLNKVFPPEVAVFEPSEAEISHTQKATLVCLATGFFPDHVELSWWVNGKEVHSGVSTDPQPLKEQPALNDSRYCLSSRLRVSATFWQNPRNHFRCQVQFYGLSENDEWTQDRAKPVTQIVSAEAWGRADCGFTSVSYQQGVLSATILYEILLGKATLYAVLVSALVLMAMVKRKDF

SEQ ID NO: 29 - protein, 115 aa, synthetic construct
KAGVTQTPRYLIKTRGQQVTLSCSPISGHRSVSWYQQTPGQGLQFLFEYFSETQRNKGNFPGRFSGRQFSNSRSEMNVSTLELGDSALYLCASSLATGGYNSPLHFGNGTRLTVT

SEQ ID NO: 30 - protein, 5 aa, synthetic construct
SGHRS

SEQ ID NO: 31 - protein, 6 aa, synthetic construct
YFSETQ

SEQ ID NO: 32 - protein, 14 aa, synthetic construct
ASSLATGGYNSPLH

SEQ ID NO: 33 - protein, 271 aa, synthetic construct
MKTFAGFSFLFLWLQLDCMSRGEDVEQSLFLSVREGDSSVINCTYTDSSSTYLYWYKQEPGAGLQLLTYIFSNMDMKQDQRLTVLLNKKDKHLSLRIADTQTGDSAIYFCAERRGNMLTFGGGTRLMVKPHIQNPDPAVYQLRDSKSSDKSVCLFTDFDSQTNVSQSKDSDVYITDKTVLDMRSMDFKSNSAVAWSNKSDFACANAFNNSIIPEDTFFPSPESSCDVKLVEKSFETDTNLNFQNLSVIGFRILLLKVAGFNLLMTLRLWSS

SEQ ID NO: 34 - protein, 109 aa, synthetic construct
GEDVEQSLFLSVREGDSSVINCTYTDSSSTYLYWYKQEPGAGLQLLTYIFSNMDMKQDQRLTVLLNKKDKHLSLRIADTQTGDSAIYFCAERRGNMLTFGGGTRLMVKP

SEQ ID NO: 35 - protein, 6 aa, synthetic construct
DSSSTY

SEQ ID NO: 36 - protein, 7 aa, synthetic construct
IFSNMDM

SEQ ID NO: 37 - protein, 9 aa, synthetic construct
AERRGNMLT

SEQ ID NO: 38 - protein, 312 aa, synthetic construct
MSISLLCCAAFPLLWAGPVNAGVTQTPKFRILKIGQSMTLQCTQDMNHNYMYWYRQDPGMGLKLIYYSVGAGITDKGEVPNGYNVSRSTTEDFPLRLELAAPSQTSVYFCASSRTSGLTDTQYFGPGTRLTVLEDLKNVFPPEVAVFEPSEAEISHTQKATLVCLATGFYPDHVELSWWVNGKEVHSGVSTDPQPLKEQPALNDSRYCLSSRLRVSATFWQNPRNHFRCQVQFYGLSENDEWTQDRAKPVTQIVSAEAWGRADCGFTSESYQQGVLSATILYEILLGKATLYAVLVSALVLMAMVKRKDSRG

SEQ ID NO: 39 - protein, 114 aa, synthetic construct
NAGVTQTPKFRILKIGQSMTLQCTQDMNHNYMYWYRQDPGMGLKLIYYSVGAGITDKGEVPNGYNVSRSTTEDFPLRLELAAPSQTSVYFCASSRTSGLTDTQYFGPGTRLTVL

SEQ ID NO: 40 - protein, 5 aa, synthetic construct
MNHNY

SEQ ID NO: 41 - protein, 6 aa, synthetic construct
SVGAGI

SEQ ID NO: 42 - protein, 13 aa, synthetic construct
ASSRTSGLTDTQY

SEQ ID NO: 43 - protein, 274 aa, synthetic construct
MEKNPLAAPLLILWFHLDCVSSILNVEQSPQSLHVQEGDSTNFTCSFPSSNFYALHWYRWETAKSPEALFVMTLNGDEKKKGRISATLNTKEGYSYLYIKGSQPEDSATYLCASADGANNLFFGTGTRLTVIPYIQNPDPAVYQLRDSKSSDKSVCLFTDFDSQTNVSQSKDSDVYITDKTVLDMRSMDFKSNSAVAWSNKSDFACANAFNNSIIPEDTFFPSPESSCDVKLVEKSFETDTNLNFQNLSVIGFRILLLKVAGFNLLMTLRLWSS

SEQ ID NO: 44 - protein, 111 aa, synthetic construct
ILNVEQSPQSLHVQEGDSTNFTCSFPSSNFYALHWYRWETAKSPEALFVMTLNGDEKKKGRISATLNTKEGYSYLYIKGSQPEDSATYLCASADGANNLFFGTGTRLTVIP

SEQ ID NO: 45 - protein, 6 aa, synthetic construct
SSNFYA

SEQ ID NO: 46 - protein, 7 aa, synthetic construct
MTLNGDE

SEQ ID NO: 47 - protein, 10 aa, synthetic construct
ASADGANNLF

SEQ ID NO: 48 - protein, 307 aa, synthetic construct
MLSLLLLLLGLGSVFSAVISQKPSRDICQRGTSLTIQCQVDSQVTMMFWYRQQPRQSLTLIATANQGSEATYESGFVIDKFPISRPNLTFSTLTVSNMSPEDSSIYLCSVGPSGTGPGYTFGSGTRLTVVEDLNKVFPPEVAVFEPSEAEISHTQKATLVCLATGFFPDHVELSWWVNGKEVHSGVSTDPQPLKEQPALNDSRYCLSSRLRVSATFWQNPRNHFRCQVQFYGLSENDEWTQDRAKPVTQIVSAEAWGRADCGFTSVSYQQGVLSATILYEILLGKATLYAVLVSALVLMAMVKRKDF

SEQ ID NO: 49 - protein, 115 aa, synthetic construct
SAVISQKPSRDICQRGTSLTIQCQVDSQVTMMFWYRQQPRQSLTLIATANQGSEATYESGFVIDKFPISRPNLTFSTLTVSNMSPEDSSIYLCSVGPSGTGPGYTFGSGTRLTVV

SEQ ID NO: 50 - protein, 5 aa, synthetic construct
SQVTM

SEQ ID NO: 51 - protein, 7 aa, synthetic construct
ANQGSEA

SEQ ID NO: 52 - protein, 12 aa, synthetic construct
SVGPSGTGPGYT

SEQ ID NO: 53 - protein, 275 aa, synthetic construct
MACPGFLWALVISTCLEFSMAQTVTQSQPEMSVQEAETVTLSCTYDTSESDYYLFWYKQPPSRQMILVIRQEAYKQQNATENRFSVNFQKAAKSFSLKISDSQLGDAAMYFCAYTNSGNTPLVFGKGTRLSVIANIQNPDPAVYQLRDSKSSDKSVCLFTDFDSQTNVSQSKDSDVYITDKTVLDMRSMDFKSNSAVAWSNKSDFACANAFNNSIIPEDTFFPSPESSCDVKLVEKSFETDTNLNFQNLSVIGFRILLLKVAGFNLLMTLRLWSS

SEQ ID NO: 54 - protein, 114 aa, synthetic construct
AQTVTQSQPEMSVQEAETVTLSCTYDTSESDYYLFWYKQPPSRQMILVIRQEAYKQQNATENRFSVNFQKAAKSFSLKISDSQLGDAAMYFCAYTNSGNTPLVFGKGTRLSVIA

SEQ ID NO: 55 - protein, 7 aa, synthetic construct
TSESDYY

SEQ ID NO: 56 - protein, 8 aa, synthetic construct
QEAYKQQN

SEQ ID NO: 57 - protein, 11 aa, synthetic construct
AYTNSGNTPLV

SEQ ID NO: 58 - protein, 312 aa, synthetic construct
MDSWTLCCVSLCILVAKHTDAGVIQSPRHEVTEMGQEVTLRCKPISGHDYLFWYRQTMMRGLELLIYFNNNVPIDDSGMPEDRFSAKMPNASFSTLKIQPSEPRDSAVYFCASKPGPRSWREGAFFGQGTRLTVVEDLNKVFPPEVAVFEPSEAEISHTQKATLVCLATGFFPDHVELSWWVNGKEVHSGVSTDPQPLKEQPALNDSRYCLSSRLRVSATFWQNPRNHFRCQVQFYGLSENDEWTQDRAKPVTQIVSAEAWGRADCGFTSVSYQQGVLSATILYEILLGKATLYAVLVSALVLMAMVKRKDF

SEQ ID NO: 59 - protein, 116 aa, synthetic construct
DAGVIQSPRHEVTEMGQEVTLRCKPISGHDYLFWYRQTMMRGLELLIYFNNNVPIDDSGMPEDRFSAKMPNASFSTLKIQPSEPRDSAVYFCASKPGPRSWREGAFFGQGTRLTVV

SEQ ID NO: 60 - protein, 5 aa, synthetic construct
SGHDY

SEQ ID NO: 61 - protein, 6 aa, synthetic construct
FNNNVP

SEQ ID NO: 62 - protein, 14 aa, synthetic construct
ASKPGPRSWREGAF

SEQ ID NO: 63 - protein, 274 aa, synthetic construct
MKTFAGFSFLFLWLQLDCMSRGEDVEQSLFLSVREGDSSVINCTYTDSSSTYLYWYKQEPGAGLQLLTYIFSNMDMKQDQRLTVLLNKKDKHLSLRIADTQTGDSAIYFCAEIEDNQGGKLIFGQGTELSVKPNIQNPDPAVYQLRDSKSSDKSVCLFTDFDSQTNVSQSKDSDVYITDKTVLDMRSMDFKSNSAVAWSNKSDFACANAFNNSIIPEDTFFPSPESSCDVKLVEKSFETDTNLNFQNLSVIGFRILLLKVAGFNLLMTLRLWSS

SEQ ID NO: 64 - protein, 112 aa, synthetic construct
GEDVEQSLFLSVREGDSSVINCTYTDSSSTYLYWYKQEPGAGLQLLTYIFSNMDMKQDQRLTVLLNKKDKHLSLRIADTQTGDSAIYFCAEIEDNQGGKLIFGQGTELSVKP

SEQ ID NO: 65 - protein, 6 aa, synthetic construct
DSSSTY

SEQ ID NO: 66 - protein, 7 aa, synthetic construct
IFSNMDM

SEQ ID NO: 67 - protein, 12 aa, synthetic construct
AEIEDNQGGKLI

SEQ ID NO: 68 - protein, 310 aa, synthetic construct
MLLLLLLLGPGSGLGAVVSQHPSRVICKSGTSVKIECRSLDFQATTMFWYRQFPKKSLMLMATSNEGSKATYEQGVEKDKFLINHASLTLSTLTVTSAHPEDSSFYICSARVPGGGADTQYFGPGTRLTVLEDLKNVFPPEVAVFEPSEAEISHTQKATLVCLATGFYPDHVELSWWVNGKEVHSGVSTDPQPLKEQPALNDSRYCLSSRLRVSATFWQNPRNHFRCQVQFYGLSENDEWTQDRAKPVTQIVSAEAWGRADCGFTSESYQQGVLSATILYEILLGKATLYAVLVSALVLMAMVKRKDSRG

SEQ ID NO: 69 - protein, 117 aa, synthetic construct
GAVVSQHPSRVICKSGTSVKIECRSLDFQATTMFWYRQFPKKSLMLMATSNEGSKATYEQGVEKDKFLINHASLTLSTLTVTSAHPEDSSFYICSARVPGGGADTQYFGPGTRLTVL

SEQ ID NO: 70 - protein, 6 aa, synthetic construct
DFQATT

SEQ ID NO: 71 - protein, 7 aa, synthetic construct
SNEGSKA

SEQ ID NO: 72 - protein, 13 aa, synthetic construct
SARVPGGGADTQY

SEQ ID NO: 73 - protein, 273 aa, synthetic construct
MKTFAGFSFLFLWLQLDCMSRGEDVEQSLFLSVREGDSSVINCTYTDSSSTYLYWYKQEPGAGLQLLTYIFSNMDMKQDQRLTVLLNKKDKHLSLRIADTQTGDSAIYFCAESIRDTDKLIFGTGTRLQVFPNIQNPDPAVYQLRDSKSSDKSVCLFTDFDSQTNVSQSKDSDVYITDKTVLDMRSMDFKSNSAVAWSNKSDFACANAFNNSIIPEDTFFPSPESSCDVKLVEKSFETDTNLNFQNLSVIGFRILLLKVAGFNLLMTLRLWSS

SEQ ID NO: 74 - protein, 111 aa, synthetic construct
GEDVEQSLFLSVREGDSSVINCTYTDSSSTYLYWYKQEPGAGLQLLTYIFSNMDMKQDQRLTVLLNKKDKHLSLRIADTQTGDSAIYFCAESIRDTDKLIFGTGTRLQVFP

SEQ ID NO: 75 - protein, 6 aa, synthetic construct
DSSSTY

SEQ ID NO: 76 - protein, 7 aa, synthetic construct
IFSNMDM

SEQ ID NO: 77 - protein, 11 aa, synthetic construct
AESIRDTDKLI

SEQ ID NO: 78 - protein, 311 aa, synthetic construct
MLLLLLLLGPGSGLGAVVSQHPSRVICKSGTSVKIECRSLDFQATTMFWYRQFPKKSLMLMATSNEGSKATYEQGVEKDKFLINHASLTLSTLTVTSAHPEDSSFYICSARDTSGTTRNEQFFGPGTRLTVLEDLKNVFPPEVAVFEPSEAEISHTQKATLVCLATGFYPDHVELSWWVNGKEVHSGVSTDPQPLKEQPALNDSRYCLSSRLRVSATFWQNPRNHFRCQVQFYGLSENDEWTQDRAKPVTQIVSAEAWGRADCGFTSESYQQGVLSATILYEILLGKATLYAVLVSALVLMAMVKRKDSRG

SEQ ID NO: 79 - protein, 118 aa, synthetic construct
GAVVSQHPSRVICKSGTSVKIECRSLDFQATTMFWYRQFPKKSLMLMATSNEGSKATYEQGVEKDKFLINHASLTLSTLTVTSAHPEDSSFYICSARDTSGTTRNEQFFGPGTRLTVL

SEQ ID NO: 80 - protein, 6 aa, synthetic construct
DFQATT

SEQ ID NO: 81 - protein, 7 aa, synthetic construct
SNEGSKA

SEQ ID NO: 82 - protein, 14 aa, synthetic construct
SARDTSGTTRNEQF

SEQ ID NO: 83 - protein, 274 aa, synthetic construct
MKTFAGFSFLFLWLQLDCMSRGEDVEQSLFLSVREGDSSVINCTYTDSSSTYLYWYKQEPGAGLQLLTYIFSNMDMKQDQRLTVLLNKKDKHLSLRIADTQTGDSAIYFCAEIPGDSSYKLIFGSGTRLLVRPDIQNPDPAVYQLRDSKSSDKSVCLFTDFDSQTNVSQSKDSDVYITDKTVLDMRSMDFKSNSAVAWSNKSDFACANAFNNSIIPEDTFFPSPESSCDVKLVEKSFETDTNLNFQNLSVIGFRILLLKVAGFNLLMTLRLWSS

SEQ ID NO: 84 - protein, 112 aa, synthetic construct
GEDVEQSLFLSVREGDSSVINCTYTDSSSTYLYWYKQEPGAGLQLLTYIFSNMDMKQDQRLTVLLNKKDKHLSLRIADTQTGDSAIYFCAEIPGDSSYKLIFGSGTRLLVRP

SEQ ID NO: 85 - protein, 6 aa, synthetic construct
DSSSTY

SEQ ID NO: 86 - protein, 7 aa, synthetic construct
IFSNMDM

SEQ ID NO: 87 - protein, 12 aa, synthetic construct
AEIPGDSSYKLI

SEQ ID NO: 88 - protein, 310 aa, synthetic construct
MASLLFFCGAFYLLGTGSMDADVTQTPRNRITKTGKRIMLECSQTKGHDRMYWYRQDPGLGLRLIYYSFDVKDINKGEISDGYSVSRQAQAKFSLSLESAIPNQTALYFCATSVTGSDTQYFGPGTRLTVLEDLKNVFPPEVAVFEPSEAEISHTQKATLVCLATGFYPDHVELSWWVNGKEVHSGVSTDPQPLKEQPALNDSRYCLSSRLRVSATFWQNPRNHFRCQVQFYGLSENDEWTQDRAKPVTQIVSAEAWGRADCGFTSESYQQGVLSATILYEILLGKATLYAVLVSALVLMAMVKRKDSRG

SEQ ID NO: 89 - protein, 112 aa, synthetic construct
DADVTQTPRNRITKTGKRIMLECSQTKGHDRMYWYRQDPGLGLRLIYYSFDVKDINKGEISDGYSVSRQAQAKFSLSLESAIPNQTALYFCATSVTGSDTQYFGPGTRLTVL

SEQ ID NO: 90 - protein, 5 aa, synthetic construct
KGHDR

SEQ ID NO: 91 - protein, 6 aa, synthetic construct
SFDVKD

SEQ ID NO: 92 - protein, 11 aa, synthetic construct
ATSVTGSDTQY

SEQ ID NO: 93 - protein, 272 aa, synthetic construct
MKTFAGFSFLFLWLQLDCMSRGEDVEQSLFLSVREGDSSVINCTYTDSSSTYLYWYKQEPGAGLQLLTYIFSNMDMKQDQRLTVLLNKKDKHLSLRIADTQTGDSAIYFCAEMKDTDKLIFGTGTRLQVFPNIQNPDPAVYQLRDSKSSDKSVCLFTDFDSQTNVSQSKDSDVYITDKTVLDMRSMDFKSNSAVAWSNKSDFACANAFNNSIIPEDTFFPSPESSCDVKLVEKSFETDTNLNFQNLSVIGFRILLLKVAGFNLLMTLRLWSS

SEQ ID NO: 94 - protein, 110 aa, synthetic construct
GEDVEQSLFLSVREGDSSVINCTYTDSSSTYLYWYKQEPGAGLQLLTYIFSNMDMKQDQRLTVLLNKKDKHLSLRIADTQTGDSAIYFCAEMKDTDKLIFGTGTRLQVFP

SEQ ID NO: 95 - protein, 6 aa, synthetic construct
DSSSTY

SEQ ID NO: 96 - protein, 7 aa, synthetic construct
IFSNMDM

SEQ ID NO: 97 - protein, 10 aa, synthetic construct
AEMKDTDKLI

SEQ ID NO: 98 - protein, 310 aa, synthetic construct
MSNQVLCCVVLCFLGANTVDGGITQSPKYLFRKEGQNVTLSCEQNLNHDAMYWYRQDPGQGLRLIYYSQIVNDFQKGDIAEGYSVSREKKESFPLTVTSAQKNPTAFYLCASTQVGTGELFFGEGSRLTVLEDLKNVFPPEVAVFEPSEAEISHTQKATLVCLATGFYPDHVELSWWVNGKEVHSGVSTDPQPLKEQPALNDSRYCLSSRLRVSATFWQNPRNHFRCQVQFYGLSENDEWTQDRAKPVTQIVSAEAWGRADCGFTSESYQQGVLSATILYEILLGKATLYAVLVSALVLMAMVKRKDSRG

SEQ ID NO: 99 - protein, 112 aa, synthetic construct
DGGITQSPKYLFRKEGQNVTLSCEQNLNHDAMYWYRQDPGQGLRLIYYSQIVNDFQKGDIAEGYSVSREKKESFPLTVTSAQKNPTAFYLCASTQVGTGELFFGEGSRLTVL

SEQ ID NO: 100 - protein, 5 aa, synthetic construct
LNHDA

SEQ ID NO: 101 - protein, 6 aa, synthetic construct
SQIVND

SEQ ID NO: 102 - protein, 11 aa, synthetic construct
ASTQVGTGELF

SEQ ID NO: 103 - protein, 272 aa, synthetic construct; identical to SEQ ID NO: 93

SEQ ID NO: 104 - protein, 110 aa, synthetic construct; identical to SEQ ID NO: 94

SEQ ID NO: 105 - protein, 6 aa, synthetic construct
DSSSTY

SEQ ID NO: 106 - protein, 7 aa, synthetic construct
IFSNMDM

SEQ ID NO: 107 - protein, 10 aa, synthetic construct
AEMKDTDKLI

SEQ ID NO: 108 - protein, 310 aa, synthetic construct; identical to SEQ ID NO: 88

SEQ ID NO: 109 - protein, 112 aa, synthetic construct; identical to SEQ ID NO: 89

SEQ ID NO: 110 - protein, 5 aa, synthetic construct
KGHDR

SEQ ID NO: 111 - protein, 6 aa, synthetic construct
SFDVKD

SEQ ID NO: 112 - protein, 11 aa, synthetic construct
ATSVTGSDTQY

SEQ ID NO: 113 - protein, 272 aa, synthetic construct
MKTFAGFSFLFLWLQLDCMSRGEDVEQSLFLSVREGDSSVINCTYTDSSSTYLYWYKQEPGAGLQLLTYIFSNMDMKQDQRLTVLLNKKDKHLSLRIADTQTGDSAIYFCAEIRDTGKLIFGQGTTLQVKPDIQNPDPAVYQLRDSKSSDKSVCLFTDFDSQTNVSQSKDSDVYITDKTVLDMRSMDFKSNSAVAWSNKSDFACANAFNNSIIPEDTFFPSPESSCDVKLVEKSFETDTNLNFQNLSVIGFRILLLKVAGFNLLMTLRLWSS

SEQ ID NO: 114 - protein, 110 aa, synthetic construct
GEDVEQSLFLSVREGDSSVINCTYTDSSSTYLYWYKQEPGAGLQLLTYIFSNMDMKQDQRLTVLLNKKDKHLSLRIADTQTGDSAIYFCAEIRDTGKLIFGQGTTLQVKP

SEQ ID NO: 115 - protein, 6 aa, synthetic construct
DSSSTY

SEQ ID NO: 116 - protein, 7 aa, synthetic construct
IFSNMDM

SEQ ID NO: 117 - protein, 10 aa, synthetic construct
AEIRDTGKLI

SEQ ID NO: 118 - protein, 310 aa, synthetic construct
MGIRLLCRVAFCFLAVGLVDVKVTQSSRYLVKRTGEKVFLECVQDMDHENMFWYRQDPGLGLRLIYFSYDVKMKEKGDIPEGYSVSREKKERFSLILESASTNQTSMYLCASSRQGTDTQYFGPGTRLTVLEDLKNVFPPEVAVFEPSEAEISHTQKATLVCLATGFYPDHVELSWWVNGKEVHSGVSTDPQPLKEQPALNDSRYCLSSRLRVSATFWQNPRNHFRCQVQFYGLSENDEWTQDRAKPVTQIVSAEAWGRADCGFTSESYQQGVLSATILYEILLGKATLYAVLVSALVLMAMVKRKDSRG

SEQ ID NO: 119 - protein, 112 aa, synthetic construct
DVKVTQSSRYLVKRTGEKVFLECVQDMDHENMFWYRQDPGLGLRLIYFSYDVKMKEKGDIPEGYSVSREKKERFSLILESASTNQTSMYLCASSRQGTDTQYFGPGTRLTVL

SEQ ID NO: 120 - protein, 5 aa, synthetic construct
MDHEN

SEQ ID NO: 121 - protein, 6 aa, synthetic construct
SYDVKM

SEQ ID NO: 122 - protein, 11 aa, synthetic construct
ASSRQGTDTQY

SEQ ID NO: 123 - protein, 272 aa, synthetic construct
MKTFAGFSFLFLWLQLDCMSRGEDVEQSLFLSVREGDSSVINCTYTDSSSTYLYWYKQEPGAGLQLLTYIFSNMDMKQDQRLTVLLNKKDKHLSLRIADTQTGDSAIYFCAERRDTDKLIFGTGTRLQVFPNIQNPDPAVYQLRDSKSSDKSVCLFTDFDSQTNVSQSKDSDVYITDKTVLDMRSMDFKSNSAVAWSNKSDFACANAFNNSIIPEDTFFPSPESSCDVKLVEKSFETDTNLNFQNLSVIGFRILLLKVAGFNLLMTLRLWSS

SEQ ID NO: 124 - protein, 110 aa, synthetic construct
GEDVEQSLFLSVREGDSSVINCTYTDSSSTYLYWYKQEPGAGLQLLTYIFSNMDMKQDQRLTVLLNKKDKHLSLRIADTQTGDSAIYFCAERRDTDKLIFGTGTRLQVFP

SEQ ID NO: 125 - protein, 6 aa, synthetic construct
DSSSTY

SEQ ID NO: 126 - protein, 7 aa, synthetic construct
IFSNMDM

SEQ ID NO: 127 - protein, 10 aa, synthetic construct
AERRDTDKLI

SEQ ID NO: 128 - protein, 308 aa, synthetic construct
MLLLLLLLGPGSGLGAVVSQHPSWVICKSGTSVKIECRSLDFQATTMFWYRQFPKQSLMLMATSNEGSKATYEQGVEKDKFLINHASLTLSTLTVTSAHPEDSSFYICSAWGANTGELFFGEGSRLTVLEDLKNVFPPEVAVFEPSEAEISHTQKATLVCLATGFYPDHVELSWWVNGKEVHSGVSTDPQPLKEQPALNDSRYCLSSRLRVSATFWQNPRNHFRCQVQFYGLSENDEWTQDRAKPVTQIVSAEAWGRADCGFTSESYQQGVLSATILYEILLGKATLYAVLVSALVLMAMVKRKDSRG

SEQ ID NO: 129 - protein, 115 aa, synthetic construct
GAVVSQHPSWVICKSGTSVKIECRSLDFQATTMFWYRQFPKQSLMLMATSNEGSKATYEQGVEKDKFLINHASLTLSTLTVTSAHPEDSSFYICSAWGANTGELFFGEGSRLTVL

SEQ ID NO: 130 - protein, 6 aa, synthetic construct
DFQATT

SEQ ID NO: 131 - protein, 7 aa, synthetic construct
SNEGSKA

SEQ ID NO: 132 - protein, 11 aa, synthetic construct
SAWGANTGELF

SEQ ID NO: 133 - protein, 276 aa, synthetic construct
MSLSSLLKVVTASLWLGPGIAQKITQTQPGMFVQEKEAVTLDCTYDTSDPSYGLFWYKQPSSGEMIFLIYQGSYDQQNATEGRYSLNFQKARKSANLVISASQLGDSAMYFCAMRGMDSSYKLIFGSGTRLLVRPDIQNPDPAVYQLRDSKSSDKSVCLFTDFDSQTNVSQSKDSDVYITDKTVLDMRSMDFKSNSAVAWSNKSDFACANAFNNSIIPEDTFFPSPESSCDVKLVEKSFETDTNLNFQNLSVIGFRILLLKVAGFNLLMTLRLWSS

SEQ ID NO: 134 - protein, 115 aa, synthetic construct
AQKITQTQPGMFVQEKEAVTLDCTYDTSDPSYGLFWYKQPSSGEMIFLIYQGSYDQQNATEGRYSLNFQKARKSANLVISASQLGDSAMYFCAMRGMDSSYKLIFGSGTRLLVRP

SEQ ID NO: 135 - protein, 7 aa, synthetic construct
TSDPSYG

SEQ ID NO: 136 - protein, 8 aa, synthetic construct
QGSYDQQN

SEQ ID NO: 137 - protein, 12 aa, synthetic construct
AMRGMDSSYKLI

SEQ ID NO: 138 - protein, 316 aa, synthetic construct
MGIRLLCRVAFCFLAVGLVDVKVTQSSRYLVKRTGEKVFLECVQDMDHENMFWYRQDPGLGLRLIYFSYDVKMKEKGDIPEGYSVSREKKERFSLILESASTNQTSMYLCATRTGQQAGSKDTDTQYFGPGTRLTVLEDLKNVFPPEVAVFEPSEAEISHTQKATLVCLATGFYPDHVELSWWVNGKEVHSGVSTDPQPLKEQPALNDSRYCLSSRLRVSATFWQNPRNHFRCQVQFYGLSENDEWTQDRAKPVTQIVSAEAWGRADCGFTSESYQQGVLSATILYEILLGKATLYAVLVSALVLMAMVKRKDSRG

SEQ ID NO: 139 - protein, 118 aa, synthetic construct
DVKVTQSSRYLVKRTGEKVFLECVQDMDHENMFWYRQDPGLGLRLIYFSYDVKMKEKGDIPEGYSVSREKKERFSLILESASTNQTSMYLCATRTGQQAGSKDTDTQYFGPGTRLTVL

SEQ ID NO: 140 - protein, 5 aa, synthetic construct
MDHEN

SEQ ID NO: 141 - protein, 6 aa, synthetic construct
SYDVKM

SEQ ID NO: 142 - protein, 17 aa, synthetic construct
ATRTGQQAGSKDTDTQY

SEQ ID NO: 143 - protein, 273 aa, synthetic construct
MKTFAGFSFLFLWLQLDCMSRGEDVEQSLFLSVREGDSSVINCTYTDSSSTYLYWYKQEPGAGLQLLTYIFSNMDMKQDQRLTVLLNKKDKHLSLRIADTQTGDSAIYFCADFLRDTDKLIFGTGTRLQVFPNIQNPDPAVYQLRDSKSSDKSVCLFTDFDSQTNVSQSKDSDVYITDKTVLDMRSMDFKSNSAVAWSNKSDFACANAFNNSIIPEDTFFPSPESSCDVKLVEKSFETDTNLNFQNLSVIGFRILLLKVAGFNLLMTLRLWSS

SEQ ID NO: 144 - protein, 111 aa, synthetic construct
GEDVEQSLFLSVREGDSSVINCTYTDSSSTYLYWYKQEPGAGLQLLTYIFSNMDMKQDQRLTVLLNKKDKHLSLRIADTQTGDSAIYFCADFLRDTDKLIFGTGTRLQVFP

SEQ ID NO: 145 - protein, 6 aa, synthetic construct
DSSSTY

SEQ ID NO: 146 - protein, 7 aa, synthetic construct
IFSNMDM

SEQ ID NO: 147 - protein, 11 aa, synthetic construct
ADFLRDTDKLI

SEQ ID NO: 148 - protein, 309 aa, synthetic construct
MLLLLLLLGPGSGLGAVVSQHPSWVICKSGTSVKIECRSLDFQATTMFWYRQFPKQSLMLMATSNEGSKATYEQGVEKDKFLINHASLTLSTLTVTSAHPEDSSFYICSARDRTSTDTQYFGPGTRLTVLEDLKNVFPPEVAVFEPSEAEISHTQKATLVCLATGFYPDHVELSWWVNGKEVHSGVSTDPQPLKEQPALNDSRYCLSSRLRVSATFWQNPRNHFRCQVQFYGLSENDEWTQDRAKPVTQIVSAEAWGRADCGFTSESYQQGVLSATILYEILLGKATLYAVLVSALVLMAMVKRKDSRG

SEQ ID NO: 149 - protein, 116 aa, synthetic construct
GAVVSQHPSWVICKSGTSVKIECRSLDFQATTMFWYRQFPKQSLMLMATSNEGSKATYEQGVEKDKFLINHASLTLSTLTVTSAHPEDSSFYICSARDRTSTDTQYFGPGTRLTVL

SEQ ID NO: 150 - protein, 6 aa, synthetic construct
DFQATT

SEQ ID NO: 151 - protein, 7 aa, synthetic construct
SNEGSKA

SEQ ID NO: 152 - protein, 12 aa, synthetic construct
SARDRTSTDTQY

SEQ ID NO: 153 - protein, 277 aa, synthetic construct
MAMLLGASVLILWLQPDWVNSQQKNDDQQVKQNSPSLSVQEGRISILNCDYTNSMFDYFLWYKKYPAEGPTFLISISSIKDKNEDGRFTVFLNKSAKHLSLHIVPSQPGDSAVYFCAVNRDDKIIFGKGTRLHILPNIQNPDPAVYQLRDSKSSDKSVCLFTDFDSQTNVSQSKDSDVYITDKTVLDMRSMDFKSNSAVAWSNKSDFACANAFNNSIIPEDTFFPSPESSCDVKLVEKSFETDTNLNFQNLSVIGFRILLLKVAGFNLLMTLRLWSS

SEQ ID NO: 154 - protein, 110 aa, synthetic construct
DQQVKQNSPSLSVQEGRISILNCDYTNSMFDYFLWYKKYPAEGPTFLISISSIKDKNEDGRFTVFLNKSAKHLSLHIVPSQPGDSAVYFCAVNRDDKIIFGKGTRLHILP

SEQ ID NO: 155 - protein, 6 aa, synthetic construct
NSMFDY

SEQ ID NO: 156 - protein, 7 aa, synthetic construct
ISSIKDK

SEQ ID NO: 157 - protein, 9 aa, synthetic construct
AVNRDDKII

SEQ ID NO: 158 - protein, 314 aa, synthetic construct
MGTSLLCWMALCLLGADHADTGVSQDPRHKITKRGQNVTFRCDPISEHNRLYWYRQTLGQGPEFLTYFQNEAQLEKSRLLSDRFSAERPKGSFSTLEIQRTEQGDSAMYLCASSSELAGGINEQFFGPGTRLTVLEDLKNVFPPEVAVFEPSEAEISHTQKATLVCLATGFYPDHVELSWWVNGKEVHSGVSTDPQPLKEQPALNDSRYCLSSRLRVSATFWQNPRNHFRCQVQFYGLSENDEWTQDRAKPVTQIVSAEAWGRADCGFTSESYQQGVLSATILYEILLGKATLYAVLVSALVLMAMVKRKDSRG

SEQ ID NO: 159 - protein, 116 aa, synthetic construct
DTGVSQDPRHKITKRGQNVTFRCDPISEHNRLYWYRQTLGQGPEFLTYFQNEAQLEKSRLLSDRFSAERPKGSFSTLEIQRTEQGDSAMYLCASSSELAGGINEQFFGPGTRLTVL

SEQ ID NO: 160 - protein, 5 aa, synthetic construct
SEHNR

SEQ ID NO: 161 - protein, 6 aa, synthetic construct
FQNEAQ

SEQ ID NO: 162 - protein, 14 aa, synthetic construct
ASSSELAGGINEQF